European Patent Specification EP 3 791 890 B1, published November 13, 2024. Title: LONG-ACTING COAGULATION FACTORS AND USES THEREOF. Applicant: OPKO BIOLOGICS LTD. The sequence listing filed with the application follows.

SEQUENCE LISTING (45 sequences)

SEQ ID NO: 1 - protein, 32 aa, Homo sapiens
DPRFQDSSSSKAPPPSLPSPSRLPGPSDTPIL

SEQ ID NO: 2 - protein, 28 aa, Homo sapiens
SSSSKAPPPSLPSPSRLPGPSDTPILPQ

SEQ ID NO: 3 - protein, 12 aa, Homo sapiens
SSSSKAPPPSLP

SEQ ID NO: 4 - protein, 28 aa, Homo sapiens
SSSSKAPPPSLPSPSRLPGPSDTPILPQ

SEQ ID NO: 5 - DNA, 25 bp, Artificial Sequence
  PCR primer for Factor VII
ctcgaggacatggtctcccaggccc

SEQ ID NO: 6 - DNA, 24 bp, Artificial Sequence
  PCR primer for Factor VII
tctagaataggtatttttccacat

SEQ ID NO: 7 - DNA, 22 bp, Artificial Sequence
  PCR primer for Factor VII
tctagaaaaaagaaatgccagc

SEQ ID NO: 8 - DNA, 32 bp, Artificial Sequence
  PCR primer for Factor VII
gcggccgcatcctcagggaaatggggctcgca

SEQ ID NO: 9 - protein, 444 aa, Homo sapiens
MVSQALRLLCLLLGLQGCLAAVFVTQEEAHGVLHRRRRANAFLEELRPGSLERECKEEQCSFEEAREIFKDAERTKLFWISYSDGDQCASSPCQNGGSCKDQLQSYICFCLPAFEGRNCETHKDDQLICVNENGGCEQYCSDHTGTKRSCRCHEGYSLLADGVSCTPTVEYPCGKIPILEKRNASKPQGRIVGGKVCPKGECPWQVLLLVNGAQLCGGTLINTIWVVSAAHCFDKIKNWRNLIAVLGEHDLSEHDGDEQSRRVAQVIIPSTYVPGTTNHDIALLRLHQPVVLTDHVVPLCLPERTFSERTLAFVRFSLVSGWGQLLDRGATALELMVLNVPRLMTQDCLQQSRKVGDSPNITEYMFCAGYSDGSKDSCKGDSGGPHATHYRGTWYLTGIVSWGQGCATVGHFGVYTRVSQYIEWLQKLMRSEPRPGVLLRAPFP

SEQ ID NO: 10 - protein, 448 aa, Homo sapiens
MVSQALRLLCLLLGLQGCLAAVFVTQEEAHGVLHRRRRANAFLEELRPGSLERECKEEQCSFEEAREIFKDAERTKLFWISYSDGDQCASSPCQNGGSCKDQLQSYICFCLPAFEGRNCETHKDDQLICVNENGGCEQYCSDHTGTKRSCRCHEGYSLLADGVSCTPTVEYPCGKIPILEKRNASKPQGRIVGGKVCPKGECPWQVLLLVNGAQLCGGTLINTIWVVSAAHCFDKIKNWRNLIAVLGEHDLSEHDGDEQSRRVAQVIIPSTYVPGTTNHDIALLRLHQPVVLTDHVVPLCLPERTFSERTLAFVRFSLVSGWGQLLDRGATALELMVLNVPRLMTQDCLQQSRKVGDSPNITEYMFCAGYSDGSKDSCKGDSGGPHATHYRGTWYLTGIVSWGQGCATVGHFGVYTRVSQYIEWLQKLMRSEPRPGVLLRAPFPGCGR

SEQ ID NO: 11 - DNA, 1356 bp, Homo sapiens
ctcgaggacatggtctcccaggccctcaggctcctctgccttctgcttgggcttcagggctgcctggctgcagtcttcgtaacccaggaggaagcccacggcgtcctgcaccggcgccggcgcgccaacgcgttcctggaggagctgcggccgggctccctggagagggagtgcaaggaggagcagtgctccttcgaggaggcccgggagatcttcaaggacgcggagaggacgaagctgttctggatttcttacagtgatggggaccagtgtgcctcaagtccatgccagaatgggggctcctgcaaggaccagctccagtcctatatctgcttctgcctccctgccttcgagggccggaactgtgagacgcacaaggatgaccagctgatctgtgtgaacgagaacggcggctgtgagcagtactgcagtgaccacacgggcaccaagcgctcctgtcggtgccacgaggggtactctctgctggcagacggggtgtcctgcacacccacagttgaatatccatgtggaaaaatacctattctagaaaaaagaaatgccagcaaaccccaaggccgaattgtggggggcaaggtgtgccccaaaggggagtgtccatggcaggtcctgttgttggtgaatggagctcagttgtgtggggggaccctgatcaacaccatctgggtggtctccgcggcccactgtttcgacaaaatcaagaactggaggaacctgatcgcggtgctgggcgagcacgacctcagcgagcacgacggggatgagcagagccggcgggtggcgcaggtcatcatccccagcacgtacgtcccgggcaccaccaaccacgacatcgcgctgctccgcctgcaccagcccgtggtcctcactgaccatgtggtgcccctctgcctgcccgaacggacgttctctgagaggacgctggccttcgtgcgcttctcattggtcagcggctggggccagctgctggaccgtggcgccacggccctggagctcatggtcctcaacgtgccccggctgatgacccaggactgcctgcagcagtcacggaaggtgggagactccccaaatatcacggagtacatgttctgtgccggctactcggatggcagcaaggactcctgcaagggggacagtggaggcccacatgccacccactaccggggcacgtggtacctgacgggcatcgtcagctggggccagggctgcgcaaccgtgggccactttggggtgtacaccagggtctcccagtacatcgagtggctgcaaaagctcatgcgctcagagccacgcccaggagtcctcctgcgagccccatttccctgaggatgcggccgc

SEQ ID NO: 12 - DNA, 1442 bp, Artificial Sequence
  CTP-modified Factor VII
ctcgaggacatggtctcccaggccctcaggctcctctgccttctgcttgggcttcagggctgcctggctgcagtcttcgtaacccaggaggaagcccacggcgtcctgcaccggcgccggcgcgccaacgcgttcctggaggagctgcggccgggctccctggagagggagtgcaaggaggagcagtgctccttcgaggaggcccgggagatcttcaaggacgcggagaggacgaagctgttctggatttcttacagtgatggggaccagtgtgcctcaagtccatgccagaatgggggctcctgcaaggaccagctccagtcctatatctgcttctgcctccctgccttcgagggccggaactgtgagacgcacaaggatgaccagctgatctgtgtgaacgagaacggcggctgtgagcagtactgcagtgaccacacgggcaccaagcgctcctgtcggtgccacgaggggtactctctgctggcagacggggtgtcctgcacacccacagttgaatatccatgtggaaaaatacctattctagaaaaaagaaatgccagcaaaccccaaggccgaattgtggggggcaaggtgtgccccaaaggggagtgtccatggcaggtcctgttgttggtgaatggagctcagttgtgtggggggaccctgatcaacaccatctgggtggtctccgcggcccactgtttcgacaaaatcaagaactggaggaacctgatcgcggtgctgggcgagcacgacctcagcgagcacgacggggatgagcagagccggcgggtggcgcaggtcatcatccccagcacgtacgtcccgggcaccaccaaccacgacatcgcgctgctccgcctgcaccagcccgtggtcctcactgaccatgtggtgcccctctgcctgcccgaacggacgttctctgagaggacgctggccttcgtgcgcttctcattggtcagcggctggggccagctgctggaccgtggcgccacggccctggagctcatggtcctcaacgtgccccggctgatgacccaggactgcctgcagcagtcacggaaggtgggagactccccaaatatcacggagtacatgttctgtgccggctactcggatggcagcaaggactcctgcaagggggacagtggaggcccacatgccacccactaccggggcacgtggtacctgaccggcatcgtgagctggggccagggctgcgccaccgtgggccacttcggcgtgtacaccagggtgtcccagtacatcgagtggctgcagaaactgatgagaagcgagcccagacccggcgtgctgctgagagcccccttccccagcagcagctccaaggcccctccccctagcctgcccagccctagcagactgcctgggcccagcgacacccccatcctgccccagtgaggatccgcggccgc

SEQ ID NO: 13 - protein, 472 aa, Artificial Sequence
  CTP-modified Factor VII
MVSQALRLLCLLLGLQGCLAAVFVTQEEAHGVLHRRRRANAFLEELRPGSLERECKEEQCSFEEAREIFKDAERTKLFWISYSDGDQCASSPCQNGGSCKDQLQSYICFCLPAFEGRNCETHKDDQLICVNENGGCEQYCSDHTGTKRSCRCHEGYSLLADGVSCTPTVEYPCGKIPILEKRNASKPQGRIVGGKVCPKGECPWQVLLLVNGAQLCGGTLINTIWVVSAAHCFDKIKNWRNLIAVLGEHDLSEHDGDEQSRRVAQVIIPSTYVPGTTNHDIALLRLHQPVVLTDHVVPLCLPERTFSERTLAFVRFSLVSGWGQLLDRGATALELMVLNVPRLMTQDCLQQSRKVGDSPNITEYMFCAGYSDGSKDSCKGDSGGPHATHYRGTWYLTGIVSWGQGCATVGHFGVYTRVSQYIEWLQKLMRSEPRPGVLLRAPFPSSSSKAPPPSLPSPSRLPGPSDTPILPQ

SEQ ID NO: 14 - DNA, 1535 bp, Artificial Sequence
  CTP-modified Factor VII
ctcgaggacatggtctcccaggccctcaggctcctctgccttctgcttgggcttcagggctgcctggctgcagtcttcgtaacccaggaggaagcccacggcgtcctgcaccggcgccggcgcgccaacgcgttcctggaggagctgcggccgggctccctggagagggagtgcaaggaggagcagtgctccttcgaggaggcccgggagatcttcaaggacgcggagaggacgaagctgttctggatttcttacagtgatggggaccagtgtgcctcaagtccatgccagaatgggggctcctgcaaggaccagctccagtcctatatctgcttctgcctccctgccttcgagggccggaactgtgagacgcacaaggatgaccagctgatctgtgtgaacgagaacggcggctgtgagcagtactgcagtgaccacacgggcaccaagcgctcctgtcggtgccacgaggggtactctctgctggcagacggggtgtcctgcacacccacagttgaatatccatgtggaaaaatacctattctagaaaaaagaaatgccagcaaaccccaaggccgaattgtggggggcaaggtgtgccccaaaggggagtgtccatggcaggtcctgttgttggtgaatggagctcagttgtgtggggggaccctgatcaacaccatctgggtggtctccgcggcccactgtttcgacaaaatcaagaactggaggaacctgatcgcggtgctgggcgagcacgacctcagcgagcacgacggggatgagcagagccggcgggtggcgcaggtcatcatccccagcacgtacgtcccgggcaccaccaaccacgacatcgcgctgctccgcctgcaccagcccgtggtcctcactgaccatgtggtgcccctctgcctgcccgaacggacgttctctgagaggacgctggccttcgtgcgcttctcattggtcagcggctggggccagctgctggaccgtggcgccacggccctggagctcatggtcctcaacgtgccccggctgatgacccaggactgcctgcagcagtcacggaaggtgggagactccccaaatatcacggagtacatgttctgtgccggctactcggatggcagcaaggactcctgcaagggggacagtggaggcccacatgccacccactaccggggcacgtggtacctgaccggcatcgtgagctggggccagggctgcgccaccgtgggccacttcggcgtgtacaccagggtgtcccagtacatcgagtggctgcagaaactgatgagaagcgagcccagacccggcgtgctgctgagagcccccttccccagcagcagctccaaggcccctccccctagcctgcccagccctagcagactgcctgggccctccgacacaccaatcctgccacagagcagctcctctaaggcccctcctccatccctgccatccccctcccggctgccaggcccctctgacacccctatcctgcctcagtgatgaaggtctggatccgcggccgc

SEQ ID NO: 15 - protein, 500 aa, Artificial Sequence
  CTP-modified Factor VII
MVSQALRLLCLLLGLQGCLAAVFVTQEEAHGVLHRRRRANAFLEELRPGSLERECKEEQCSFEEAREIFKDAERTKLFWISYSDGDQCASSPCQNGGSCKDQLQSYICFCLPAFEGRNCETHKDDQLICVNENGGCEQYCSDHTGTKRSCRCHEGYSLLADGVSCTPTVEYPCGKIPILEKRNASKPQGRIVGGKVCPKGECPWQVLLLVNGAQLCGGTLINTIWVVSAAHCFDKIKNWRNLIAVLGEHDLSEHDGDEQSRRVAQVIIPSTYVPGTTNHDIALLRLHQPVVLTDHVVPLCLPERTFSERTLAFVRFSLVSGWGQLLDRGATALELMVLNVPRLMTQDCLQQSRKVGDSPNITEYMFCAGYSDGSKDSCKGDSGGPHATHYRGTWYLTGIVSWGQGCATVGHFGVYTRVSQYIEWLQKLMRSEPRPGVLLRAPFPSSSSKAPPPSLPSPSRLPGPSDTPILPQSSSSKAPPPSLPSPSRLPGPSDTPILPQ

SEQ ID NO: 16 - DNA, 1404 bp, Homo sapiens
gcgatcgccatgcagcgcgtgaacatgatcatggcagaatcaccaggcctcatcaccattgccttttaggatatctactcagtgctgaatgtacagtttttcttgatcatgaaaacgccaacaaaattctgaatcggccaaagaggtataattcaggtaaattggaagagtttgttcaagggaaccttgagagagaatgtatggaagaaaagtgtagttttgaagaagcacgagaagtttttgaaaacactgaaagaacaactgaattttggaagcagtatgttgatggagatcagtgtgagtccaatccatgtttaaatggcggcagttgcaaggatgacattaattcctatgaatgttggtgtccctttggatttgaaggaaagaactgtgaattagatgtaacatgtaacattaagaatggcagatgcgagcagttttgtaaaaatagtgctgataacaaggtggtttgctcctgtactgagggatatcgacttgcagaaaaccagaagtcctgtgaaccagcagtgccatttccatgtggaagagtttctgtttcacaaacttctaagctcacccgtgctgagactgtttttcctgatgtggactatgtaaattctactgaagctgaaaccattttggataacatcactcaaagcacccaatcatttaatgacttcactcgagttgttggtggagaagatgccaaaccaggtcaattcccttggcaggttgttttgaatggtaaagttgatgcattctgtggaggctctatcgttaatgaaaaatggattgtaactgctgcccactgtgttgaaactggtgttaaaattacagttgtcgcaggtgaacataatattgaggagacagaacatacagagcaaaagcgaaatgtgattcgaattattcctcaccacaactacaatgcagctattaataagtacaaccatgacattgcccttctggaactggacgaacccttagtgctaaacagctacgttacacctatttgcattgctgacaaggaatacacgaacatcttcctcaaatttggatctggctatgtaagtggctggggaagagtcttccacaaagggagatcagctttagttctccagtaccttagagttccacttgttgaccgagccacatgtcttcgatctacaaagttcaccatctataacaacatgttctgtgctggcttccatgaaggaggtagagattcatgtcaaggagatagtgggggaccccatgttactgaagtggaagggaccagtttcttaactggaattattagctggggtgaagagtgtgcaatgaaaggcaaatatggaatatataccaaggtatcccggtatgtcaactggattaaggaaaaaacaaagctcacttgaacgcggccgc

SEQ ID NO: 17 - protein, 461 aa, Homo sapiens
MQRVNMIMAESPGLITICLLGYLLSAECTVFLDHENANKILNRPKRYNSGKLEEFVQGNLERECMEEKCSFEEAREVFENTERTTEFWKQYVDGDQCESNPCLNGGSCKDDINSYECWCPFGFEGKNCELDVTCNIKNGRCEQFCKNSADNKVVCSCTEGYRLAENQKSCEPAVPFPCGRVSVSQTSKLTRAETVFPDVDYVNSTEAETILDNITQSTQSFNDFTRVVGGEDAKPGQFPWQVVLNGKVDAFCGGSIVNEKWIVTAAHCVETGVKITVVAGEHNIEETEHTEQKRNVIRIIPHHNYNAAINKYNHDIALLELDEPLVLNSYVTPICIADKEYTNIFLKFGSGYVSGWGRVFHKGRSALVLQYLRVPLVDRATCLRSTKFTIYNNMFCAGFHEGGRDSCQGDSGGPHVTEVEGTSFLTGIISWGEECAMKGKYGIYTKVSRYVNWIKEKTKLT

SEQ ID NO: 18 - DNA, 1502 bp, Artificial Sequence
  CTP-modified Factor IX
gcgatcgccatgcagcgcgtgaacatgatcatggcagaatcaccaggcctcatcaccatctgccttttaggatatctactcagtgctgaatgtacagtttttcttgatcatgaaaacgccaacaaaattctgaatcggccaaagaggtataattcaggtaaattggaagagtttgttcaagggaaccttgagagagaatgtatggaagaaaagtgtagttttgaagaagcacgagaagtttttgaaaacactgaaagaacaactgaattttggaagcagtatgttgatggagatcagtgtgagtccaatccatgtttaaatggcggcagttgcaaggatgacattaattcctatgaatgttggtgtccctttggatttgaaggaaagaactgtgaattagatgtaacatgtaacattaagaatggcagatgcgagcagttttgtaaaaatagtgctgataacaaggtggtttgctcctgtactgagggatatcgacttgcagaaaaccagaagtcctgtgaaccagcagtgccatttccatgtggaagagtttctgtttcacaaacttctaagctcacccgtgctgagactgtttttcctgatgtggactatgtaaattctactgaagctgaaaccattttggataacatcactcaaagcacccaatcatttaatgacttcactcgagttgttggtggagaagatgccaaaccaggtcaattcccttggcaggttgttttgaatggtaaagttgatgcattctgtggaggctctatcgttaatgaaaaatggattgtaactgctgcccactgtgttgaaactggtgttaaaattacagttgtcgcaggtgaacataatattgaggagacagaacatacagagcaaaagcgaaatgtgattcgaattattcctcaccacaactacaatgcagctattaataagtacaaccatgacattgcccttctggaactggacgaacccttagtgctaaacagctacgttacacctatttgcattgctgacaaggaatacacgaacatcttcctcaaatttggatctggctatgtaagtggctggggaagagtcttccacaaagggagatcagctttagttcttcagtaccttagagttccacttgttgaccgagccacatgtcttcgatctacaaagttcaccatctataacaacatgttctgtgctggcttccatgaaggaggtagagattcatgtcaaggagatagtgggggaccccatgttactgaagtggaagggaccagtttcttaactggaattattagctggggtgaagagtgtgcaatgaaaggcaaatatggaatatataccaaggtatcccggtatgtcaactggattaaggaaaaaacaaagctcactagctccagcagcaaggcccctcccccgagcctgccctccccaagcaggctgcctgggccctccgacacaccaatcctgccacagtgatgaaggtctggatccgcggccgc

SEQ ID NO: 19 - protein, 489 aa, Artificial Sequence
  CTP-modified Factor IX
MQRVNMIMAESPGLITICLLGYLLSAECTVFLDHENANKILNRPKRYNSGKLEEFVQGNLERECMEEKCSFEEAREVFENTERTTEFWKQYVDGDQCESNPCLNGGSCKDDINSYECWCPFGFEGKNCELDVTCNIKNGRCEQFCKNSADNKVVCSCTEGYRLAENQKSCEPAVPFPCGRVSVSQTSKLTRAETVFPDVDYVNSTEAETILDNITQSTQSFNDFTRVVGGEDAKPGQFPWQVVLNGKVDAFCGGSIVNEKWIVTAAHCVETGVKITVVAGEHNIEETEHTEQKRNVIRIIPHHNYNAAINKYNHDIALLELDEPLVLNSYVTPICIADKEYTNIFLKFGSGYVSGWGRVFHKGRSALVLQYLRVPLVDRATCLRSTKFTIYNNMFCAGFHEGGRDSCQGDSGGPHVTEVEGTSFLTGIISWGEECAMKGKYGIYTKVSRYVNWIKEKTKLTSSSSKAPPPSLPSPSRLPGPSDTPILPQ

SEQ ID NO: 20 - DNA, 1585 bp, Artificial Sequence
  CTP-modified Factor IX
gcgatcgccatgcagcgcgtgaacatgatcatggcagaatcaccaggcctcatcaccatctgccttttaggatatctactcagtgctgaatgtacagtttttcttgatcatgaaaacgccaacaaaattctgaatcggccaaagaggtataattcaggtaaattggaagagtttgttcaagggaaccttgagagagaatgtatggaagaaaagtgtagttttgaagaagcacgagaagtttttgaaaacactgaaagaacaactgaattttggaagcagtatgttgatggagatcagtgtgagtccaatccatgtttaaatggcggcagttgcaaggatgacattaattcctatgaatgttggtgtccctttggatttgaaggaaagaactgtgaattagatgtaacatgtaacattaagaatggcagatgcgagcagttttgtaaaaatagtgctgataacaaggtggtttgctcctgtactgagggatatcgacttgcagaaaaccagaagtcctgtgaaccagcagtgccatttccatgtggaagagtttctgtttcacaaacttctaagctcacccgtgctgagactgtttttcctgatgtggactatgtaaattctactgaagctgaaaccattttggataacatcactcaaagcacccaatcatttaatgacttcactcgagttgttggtggagaagatgccaaaccaggtcaattcccttggcaggttgttttgaatggtaaagttgatgcattctgtggaggctctatcgttaatgaaaaatggattgtaactgctgcccactgtgttgaaactggtgttaaaattacagttgtcgcaggtgaacataatattgaggagacagaacatacagagcaaaagcgaaatgtgattcgaattattcctcaccacaactacaatgcagctattaataagtacaaccatgacattgcccttctggaactggacgaacccttagtgctaaacagctacgttacacctatttgcattgctacaaggaatacacgaacatcttcctcaaatttggatctggctatgtaagtggctggggaagagtcttccacaaagggagatcagctttagttcttcagtaccttagagttccacttgttgaccgagccacatgtcttcgatctacaaagttcaccatctataacaacatgttctgtgctggcttccatgaaggaggtagagattcatgtcaaggagatagtgggggaccccatgttactgaagtggaagggaccagtttcttaactggaattattagctggggtgaagagtgtgcaatgaaaggcaaatatggaatatataccaaggtatcccggtatgtcaactggattaaggaaaaaacaaagctcactagctccagcagcaaggcccctcccccgagcctgccctccccaagcaggctgcctgggccctccgacacaccaatcctgccacagagcagctcctctaaggcccctcctccatccctgccatccccctcccggctgcctggcccctctgacacccctatcctgcctcagtgatgaaggtctggatccgcggccgc

SEQ ID NO: 21 - protein, 517 aa, Artificial Sequence
  CTP-modified Factor IX
MQRVNMIMAESPGLITICLLGYLLSAECTVFLDHENANKILNRPKRYNSGKLEEFVQGNLERECMEEKCSFEEAREVFENTERTTEFWKQYVDGDQCESNPCLNGGSCKDDINSYECWCPFGFEGKNCELDVTCNIKNGRCEQFCKNSADNKVVCSCTEGYRLAENQKSCEPAVPFPCGRVSVSQTSKLTRAETVFPDVDYVNSTEAETILDNITQSTQSFNDFTRVVGGEDAKPGQFPWQVVLNGKVDAFCGGSIVNEKWIVTAAHCVETGVKITVVAGEHNIEETEHTEQKRNVIRIIPHHNYNAAINKYNHDIALLELDEPLVLNSYVTPICIADKEYTNIFLKFGSGYVSGWGRVFHKGRSALVLQYLRVPLVDRATCLRSTKFTIYNNMFCAGFHEGGRDSCQGDSGGPHVTEVEGTSFLTGIISWGEECAMKGKYGIYTKVSRYVNWIKEKTKLTSSSSKAPPPSLPSPSRLPGPSDTPILPQSSSSKAPPPSLPSPSRLPGPSDTPILPQ

SEQ ID NO: 22 - DNA, 2413 bp, Homo sapiens
tctagagtcgaccccgccatggagctgaggccctggttgctatgggtggtagcagcaacaggaaccttggtcctgctagcagctgatgctcagggccagaaggtcttcaccaacacgtgggctgtgcgcatccctggaggcccagcggtggccaacagtgtggcacggaagcatgggttcctcaacctgggccagatcttcggggactattaccacttctggcatcgaggagtgacgaagcggtccctgtcgcctcaccgcccgcggcacagccggctgcagagggagcctcaagtacagtggctggaacagcaggtggcaaagcgacggactaaacgggacgtgtaccaggagcccacagaccccaagtttcctcagcagtggtacctgtctggtgtcactcagcgggacctgaatgtgaaggcggcctgggcgcagggctacacagggcacggcattgtggtctccattctggacgatggcatcgagaagaaccacccggacttggcaggcaattatgatcctggggccagttttgatgtcaatgaccaggaccctgacccccagcctcggtacacacagatgaatgacaacaggcacggcacacggtgtgcgggggaagtggctgcggtggccaacaacggtgtctgtggtgtaggtgtggcctacaacgcccgcattggaggggtgcgcatgctggatggcgaggtgacagatgcagtggaggcacgctcgctgggcctgaaccccaaccacatccacatctacagtgccagctggggccccgaggatgacggcaagacagtggatgggccagcccgcctcgccgaggaggccttcttccgtggggttagccagggccgaggggggctgggctccatctttgtctgggcctcggggaacgggggccgggaacatgacagctgcaactgcgacggctacaccaacagtatctacacgctgtccatcagcagcgccacgcagtttggcaacgtgccgtggtacagcgaggcctgctcgtccacactggccacgacctacagcagtggcaaccagaatgagaagcagatcgtgacgactgacttgcggcagaagtgcacggagtctcacacgggcacctcagcctctgcccccttagcagccggcatcattgctctcaccctggaggccaataagaacctcacatggcgggacatgcaacacctggtggtacagacctcgaagccagcccacctcaatgccaacgactgggccaccaatggtgtgggccggaaagtgagccactcatatggctacgggcttttggacgcaggcgccatggtggccctggcccagaattggaccacagtggccccccagcggaagtgcatcatcgacatcctcaccgagcccaaagacatcgggaaacggctcgaggtgcggaagaccgtgaccgcgtgcctgggcgagcccaaccacatcactcggctggagcacgctcaggcgcggctcaccctgtcctataatcgccgtggcgacctggccatccacctggtcagccccatgggcacccgctccaccctgctggcagccaggccacatgactactccgcagatgggtttaatgactgggccttcatgacaactcattcctgggatgaggatccctctggcgagtgggtcctagagattgaaaacaccagcgaagccaacaactatgggacgctgaccaagttcaccctcgtactctatggcaccgcccctgaggggctgcccgtacctccagaaagcagtggctgcaagaccctcacgtccagtcaggcctgtgtggtgtgcgaggaaggcttctccctgcaccagaagagctgtgtccagcactgccctccaggcttcgccccccaagtcctcgatacgcactatagcaccgagaatgacgtggagaccatccgggccagcgtctgcgccccctgccacgcctcatgtgccacatgccaggggccggccctgacagactgcctcagctgccccagccacgcctccttggaccctgtggagcagacttgctcccggcaaagccagagcagccgagagtccccgccacagcagcagccacctcggctgcccccggaggtggaggcggggcaacggctgcgggcagggctgctgccctcacacctgcctgaggtggtggccggcctcagctgcgccttcatcgtgctggtcttcgtcactgtcttcctggtcctgcagctgcgctctggctttagttttcggggggtgaaggtgtacaccatggaccgtggcctcatctcctacaaggggctgccccctgaagcctggcaggaggagtgcccgtctgactcagaagaggacgagggccggggcgagaggaccgcctttatcaaagaccagagcgccctctgaacgcggccgc

SEQ ID NO: 23 - protein, 794 aa, Homo sapiens
MELRPWLLWVVAATGTLVLLAADAQGQKVFTNTWAVRIPGGPAVANSVARKHGFLNLGQIFGDYYHFWHRGVTKRSLSPHRPRHSRLQREPQVQWLEQQVAKRRTKRDVYQEPTDPKFPQQWYLSGVTQRDLNVKAAWAQGYTGHGIVVSILDDGIEKNHPDLAGNYDPGASFDVNDQDPDPQPRYTQMNDNRHGTRCAGEVAAVANNGVCGVGVAYNARIGGVRMLDGEVTDAVEARSLGLNPNHIHIYSASWGPEDDGKTVDGPARLAEEAFFRGVSQGRGGLGSIFVWASGNGGREHDSCNCDGYTNSIYTLSISSATQFGNVPWYSEACSSTLATTYSSGNQNEKQIVTTDLRQKCTESHTGTSASAPLAAGIIALTLEANKNLTWRDMQHLVVQTSKPAHLNANDWATNGVGRKVSHSYGYGLLDAGAMVALAQNWTTVAPQRKCIIDILTEPKDIGKRLEVRKTVTACLGEPNHITRLEHAQARLTLSYNRRGDLAIHLVSPMGTRSTLLAARPHDYSADGFNDWAFMTTHSWDEDPSGEWVLEIENTSEANNYGTLTKFTLVLYGTAPEGLPVPPESSGCKTLTSSQACVVCEEGFSLHQKSCVQHCPPGFAPQVLDTHYSTENDVETIRASVCAPCHASCATCQGPALTDCLSCPSHASLDPVEQTCSRQSQSSRESPPQQQPPRLPPEVEAGQRLRAGLLPSHLPEVVAGLSCAFIVLVFVTVFLVLQLRSGFSFRGVKVYTMDRGLISYKGLPPEAWQEECPSDSEEDEGRGERTAFIKDQSAL

SEQ ID NO: 24 - DNA, 1621 bp, Artificial Sequence
  CTP-modified Factor VII
ctcgaggacatggtctcccaggccctcaggctcctctgccttctgcttgggcttcagggctgcctggctgcagtcttcgtaacccaggaggaagcccacggcgtcctgcaccggcgccggcgcgccaacgcgttcctggaggagctgcggccgggctccctggagagggagtgcaaggaggagcagtgctccttcgaggaggcccgggagatcttcaaggacgcggagaggacgaagctgttctggatttcttacagtgatggggaccagtgtgcctcaagtccatgccagaatgggggctcctgcaaggaccagctccagtcctatatctgcttctgcctccctgccttcgagggccggaactgtgagacgcacaaggatgaccagctgatctgtgtgaacgagaacggcggctgtgagcagtactgcagtgaccacacgggcaccaagcgctcctgtcggtgccacgaggggtactctctgctggcagacggggtgtcctgcacacccacagttgaatatccatgtggaaaaatacctattctagaaaaaagaaatgccagcaaaccccaaggccgaattgtggggggcaaggtgtgccccaaaggggagtgtccatggcaggtcctgttgttggtgaatggagctcagttgtgtggggggaccctgatcaacaccatctgggtggtctccgcggcccactgtttcgacaaaatcaagaactggaggaacctgatcgcggtgctgggcgagcacgacctcagcgagcacgacggggatgagcagagccggcgggtggcgcaggtcatcatccccagcacgtacgtcccgggcaccaccaaccacgacatcgcgctgctccgcctgcaccagcccgtggtcctcactgaccatgtggtgcccctctgcctgcccgaacggacgttctctgagaggacgctggccttcgtgcgcttctcattggtcagcggctggggccagctgctggaccgtggcgccacggccctggagctcatggtcctcaacgtgccccggctgatgacccaggactgcctgcagcagtcacggaaggtgggagactccccaaatatcacggagtacatgttctgtgccggctactcggatggcagcaaggactcctgcaagggggacagtggaggcccacatgccacccactaccggggcacgtggtacctgaccggcatcgtgagctggggccagggctgcgccaccgtgggccacttcggcgtgtacaccagggtgtcccagtacatcgagtggctgcagaaactgatgagaagcgagcccagacccggcgtgctgctgagagcccccttccccagcagcagctccaaggcccctccccctagcctgcccagccctagcagactgcctgggcccagtgacacccctatcctgcctcagtccagctccagcaaggccccaccccctagcctgccttctccttctcggctgcctggccccagcgatactccaattctgccccagtcctccagcagtaaggctccccctccatctctgccatcccccagcagactgccaggcccttctgatacacccatcctcccacagtgatgaggatccgcggccgcttaattaa

SEQ ID NO: 25 - protein, 528 aa, Artificial Sequence
  CTP-modified Factor VII
MVSQALRLLCLLLGLQGCLAAVFVTQEEAHGVLHRRRRANAFLEELRPGSLERECKEEQCSFEEAREIFKDAERTKLFWISYSDGDQCASSPCQNGGSCKDQLQSYICFCLPAFEGRNCETHKDDQLICVNENGGCEQYCSDHTGTKRSCRCHEGYSLLADGVSCTPTVEYPCGKIPILEKRNASKPQGRIVGGKVCPKGECPWQVLLLVNGAQLCGGTLINTIWVVSAAHCFDKIKNWRNLIAVLGEHDLSEHDGDEQSRRVAQVIIPSTYVPGTTNHDIALLRLHQPVVLTDHVVPLCLPERTFSERTLAFVRFSLVSGWGQLLDRGATALELMVLNVPRLMTQDCLQQSRKVGDSPNITEYMFCAGYSDGSKDSCKGDSGGPHATHYRGTWYLTGIVSWGQGCATVGHFGVYTRVSQYIEWLQKLMRSEPRPGVLLRAPFPSSSSKAPPPSLPSPSRLPGPSDTPILPQSSSSKAPPPSLPSPSRLPGPSDTPILPQSSSSKAPPPSLPSPSRLPGPSDTPILPQ

SEQ ID NO: 26 - DNA, 1607 bp, Artificial Sequence
  CTP-modified Factor VII
ctcgaggacatggtctcccaggccctcaggctcctctgccttctgcttgggcttcagggctgcctggctgcagtcttcgtaacccaggaggaagcccacggcgtcctgcaccggcgccggcgcgccaacgcgttcctggaggagctgcggccgggctccctggagagggagtgcaaggaggagcagtgctccttcgaggaggcccgggagatcttcaaggacgcggagaggacgaagctgttctggatttcttacagtgatggggaccagtgtgcctcaagtccatgccagaatgggggctcctgcaaggaccagctccagtcctatatctgcttctgcctccctgccttcgagggccggaactgtgagacgcacaaggatgaccagctgatctgtgtgaacgagaacggcggctgtgagcagtactgcagtgaccacacgggcaccaagcgctcctgtcggtgccacgaggggtactctctgctggcagacggggtgtcctgcacacccacagttgaatatccatgtggaaaaatacctattctagaaaaaagaaatgccagcaaaccccaaggccgaattgtggggggcaaggtgtgccccaaaggggagtgtccatggcaggtcctgttgttggtgaatggagctcagttgtgtggggggaccctgatcaacaccatctgggtggtctccgcggcccactgtttcgacaaaatcaagaactggaggaacctgatcgcggtgctgggcgagcacgacctcagcgagcacgacggggatgagcagagccggcgggtggcgcaggtcatcatccccagcacgtacgtcccgggcaccaccaaccacgacatcgcgctgctccgcctgcaccagcccgtggtcctcactgaccatgtggtgcccctctgcctgcccgaacggacgttctctgagaggacgctggccttcgtgcgcttctcattggtcagcggctggggccagctgctggaccgtggcgccacggccctggagctcatggtcctcaacgtgccccggctgatgacccaggactgcctgcagcagtcacggaaggtgggagactccccaaatatcacggagtacatgttctgtgccggctactcggatggcagcaaggactcctgcaagggggacagtggaggcccacatgccacccactaccggggcacgtggtacctgaccggcatcgtgagctggggccagggctgcgccaccgtgggccacttcggcgtgtacaccagggtgtcccagtacatcgagtggctgcagaaactgatgagaagcgagcccagacccggcgtgctgctgagagcccccttccccagcagcagctccaaggcccctccccctagcctgcccagccctagcagactgcctgggcccagtgacacccctatcctgcctcagtccagctccagcaaggccccaccccctagcctgccttctccttctcggctgcctggccccagcgatactccaattctgccccagtcctccagcagtaaggctccccctccatctctgccatcccccagcagactgccaggcccttctgatacacccatcctcccacagtgatgaggatccgc

SEQ ID NO: 27 - protein, 532 aa, Artificial Sequence
  CTP-modified Factor VII
LEDMVSQALRLLCLLLGLQGCLAAVFVTQEEAHGVLHRRRRANAFLEELRPGSLERECKEEQCSFEEAREIFKDAERTKLFWISYSDGDQCASSPCQNGGSCKDQLQSYICFCLPAFEGRNCETHKDDQLICVNENGGCEQYCSDHTGTKRSCRCHEGYSLLADGVSCTPTVEYPCGKIPILEKRNASKPQGRIVGGKVCPKGECPWQVLLLVNGAQLCGGTLINTIWVVSAAHCFDKIKNWRNLIAVLGEHDLSEHDGDEQSRRVAQVIIPSTYVPGTTNHDIALLRLHQPVVLTDHVVPLCLPERTFSERTLAFVRFSLVSGWGQLLDRGATALELMVLNVPRLMTQDCLQQSRKVGDSPNITEYMFCAGYSDGSKDSCKGDSGGPHATHYRGTWYLTGIVSWGQGCATVGHFGVYTRVSQYIEWLQKLMRSEPRPGVLLRAPFPSSSSKAPPPSLPSPSRLPGPSDTPILPQSSSSKAPPPSLPSPSRLPGPSDTPILPQSSSSKAPPPSLPSPSRLPGPSDTPILPQG

SEQ ID NO: 28 - DNA, 1775 bp, Artificial Sequence
  CTP-modified Factor VII
ctcgaggacatggtctcccaggccctcaggctcctctgccttctgcttgggcttcagggctgcctggctgcagtcttcgtaacccaggaggaagcccacggcgtcctgcaccggcgccggcgcgccaacgcgttcctggaggagctgcggccgggctccctggagagggagtgcaaggaggagcagtgctccttcgaggaggcccgggagatcttcaaggacgcggagaggacgaagctgttctggatttcttacagtgatggggaccagtgtgcctcaagtccatgccagaatgggggctcctgcaaggaccagctccagtcctatatctgcttctgcctccctgccttcgagggccggaactgtgagacgcacaaggatgaccagctgatctgtgtgaacgagaacggcggctgtgagcagtactgcagtgaccacacgggcaccaagcgctcctgtcggtgccacgaggggtactctctgctggcagacggggtgtcctgcacacccacagttgaatatccatgtggaaaaatacctattctagaaaaaagaaatgccagcaaaccccaaggccgaattgtggggggcaaggtgtgccccaaaggggagtgtccatggcaggtcctgttgttggtgaatggagctcagttgtgtggggggaccctgatcaacaccatctgggtggtctccgcggcccactgtttcgacaaaatcaagaactggaggaacctgatcgcggtgctgggcgagcacgacctcagcgagcacgacggggatgagcagagccggcgggtggcgcaggtcatcatccccagcacgtacgtcccgggcaccaccaaccacgacatcgcgctgctccgcctgcaccagcccgtggtcctcactgaccatgtggtgcccctctgcctgcccgaacggacgttctctgagaggacgctggccttcgtgcgcttctcattggtcagcggctggggccagctgctggaccgtggcgccacggccctggagctcatggtcctcaacgtgccccggctgatgacccaggactgcctgcagcagtcacggaaggtgggagactccccaaatatcacggagtacatgttctgtgccggctactcggatggcagcaaggactcctgcaagggggacagtggaggcccacatgccacccactaccggggcacgtggtacctgaccggcatcgtgagctggggccagggctgcgccaccgtgggccacttcggcgtgtacaccagggtgtcccagtacatcgagtggctgcagaaactgatgagaagcgagcccagacccggcgtgctgctgagagcccccttccccagcagcagctccaaggcccctccccctagcctgcccagccctagcagactgcctgggccctctgacacccctatcctgcctcagtccagctcctctaaggctccaccaccttccctgcctagcccttcaagactgccaggccctagcgatacaccaattctgccccagtcctccagcagcaaggctcccccacctagcctgccttctccatcaaggctgcctggcccatccgataccccaattttgcctcagagcagctctagcaaggcacctccccccagtctgccctctccaagcagactccctggcccttcagacactccaatcctcccacagtcctctagctctaaagctccacctcccagcctgcccagccctagtagactccccggaccttctgatacccccatcttgccccagtgatgaggatccgc

SEQ ID NO: 29 - protein, 589 aa, Artificial Sequence
  CTP-modified Factor VII
LEDMVSQALRLLCLLLGLQGCLAAVFVTQEEAHGVLHRRRRANAFLEELRPGSLERECKEEQCSFEEAREIFKDAERTKLFWISYSDGDQCASSPCQNGGSCKDQLQSYICFCLPAFEGRNCETHKDDQLICVNENGGCEQYCSDHTGTKRSCRCHEGYSLLADGVSCTPTVEYPCGKIPILEKRNASKPQGRIVGGKVCPKGECPWQVLLLVNGAQLCGGTLINTIWVVSAAHCFDKIKNWRNLIAVLGEHDLSEHDGDEQSRRVAQVIIPSTYVPGTTNHDIALLRLHQPVVLTDHVVPLCLPERTFSERTLAFVRFSLVSGWGQLLDRGATALELMVLNVPRLMTQDCLQQSRKVGDSPNITEYMFCAGYSDGSKDSCKGDSGGPHATHYRGTWYLTGIVSWGQGCATVGHFGVYTRVSQYIEWLQKLMRSEPRPGVLLRAPFPSSSSKAPPPSLPSPSRLPGPSDTPILPQSSSSKAPPPSLPSPSRLPGPSDTPILPQSSSSKAPPPSLPSPSRLPGPSDTPILPQSSSSKAPPPSLPSPSRLPGPSDTPILPQSSSSKAPPPSLPSPSRLPGPSDTPILPQGS

SEQ ID NO: 30 - DNA, 1673 bp, Artificial Sequence
  CTP-modified Factor IX
tctagagtcgaccccgccatgcagcgcgtgaacatgatcatggcagaatcaccaggcctcatcaccatctgccttttaggatatctactcagtgctgaatgtacagtttttcttgatcatgaaaacgccaacaaaattctgaatcggccaaagaggtataattcaggtaaattggaagagtttgttcaagggaaccttgagagagaatgtatggaagaaaagtgtagttttgaagaagcacgagaagtttttgaaaacactgaaagaacaactgaattttggaagcagtatgttgatggagatcagtgtgagtccaatccatgtttaaatggcggcagttgcaaggatgacattaattcctatgaatgttggtgtccctttggatttgaaggaaagaactgtgaattagatgtaacatgtaacattaagaatggcagatgcgagcagttttgtaaaaatagtgctgataacaaggtggtttgctcctgtactgagggatatcgacttgcagaaaaccagaagtcctgtgaaccagcagtgccatttccatgtggaagagtttctgtttcacaaacttctaagctcacccgtgctgaggcagtttttcctgatgtggactatgtaaattctactgaagctgaaaccattttggataacatcactcaaagcacccaatcatttaatgacttcactcgagttgttggtggagaagatgccaaaccaggtcaattcccttggcaggttgttttgaatggtaaagttgatgcattctgtggaggctctatcgttaatgaaaaatggattgtaactgctgcccactgtgttgaaactggtgttaaaattacagttgtcgcaggtgaacataatattgaggagacagaacatacagagcaaaagcgaaatgtgattcgaattattcctcaccacaactacaatgcagctattaataagtacaaccatgacattgcccttctggaactggacgaacccttagtgctaaacagctacgttacacctatttgcattgctgacaaggaatacacgaacatcttcctcaaatttggatctggctatgtaagtggctggggaagagtcttccacaaagggagatcagctttagttcttcagtaccttagagttccacttgttgaccgagccacatgtcttcgatctacaaagttcaccatctataacaacatgttctgtgctggcttccatgaaggaggtagagattcatgtcaaggagatagtgggggaccccatgttactgaagtggaagggaccagtttcttaactggaattattagctggggtgaagagtgtgcaatgaaaggcaaatatggaatatataccaaggtatcccggtatgtcaactggattaaggaaaaaacaaagctcactagctccagcagcaaggcccctcccccgagcctgccctccccaagcaggctgcctgggcccagtgacacccctatcctgcctcagtccagctccagcaaggccccaccccctagcctgccttctccttctcggctgcctggccccagcgatactccaattctgccccagtcctccagcagtaaggctccccctccatctctgccatcccccagcagactgccaggcccttctgatacacccatcctcccacagtgatgaggatccgcggccgc

SEQ ID NO: 31 - protein, 545 aa, Artificial Sequence
  CTP-modified Factor IX
MQRVNMIMAESPGLITICLLGYLLSAECTVFLDHENANKILNRPKRYNSGKLEEFVQGNLERECMEEKCSFEEAREVFENTERTTEFWKQYVDGDQCESNPCLNGGSCKDDINSYECWCPFGFEGKNCELDVTCNIKNGRCEQFCKNSADNKVVCSCTEGYRLAENQKSCEPAVPFPCGRVSVSQTSKLTRAEAVFPDVDYVNSTEAETILDNITQSTQSFNDFTRVVGGEDAKPGQFPWQVVLNGKVDAFCGGSIVNEKWIVTAAHCVETGVKITVVAGEHNIEETEHTEQKRNVIRIIPHHNYNAAINKYNHDIALLELDEPLVLNSYVTPICIADKEYTNIFLKFGSGYVSGWGRVFHKGRSALVLQYLRVPLVDRATCLRSTKFTIYNNMFCAGFHEGGRDSCQGDSGGPHVTEVEGTSFLTGIISWGEECAMKGKYGIYTKVSRYVNWIKEKTKLTSSSSKAPPPSLPSPSRLPGPSDTPILPQSSSSKAPPPSLPSPSRLPGPSDTPILPQSSSSKAPPPSLPSPSRLPGPSDTPILPQ

SEQ ID NO: 32 - DNA, 1757 bp, Artificial Sequence
  CTP-modified Factor IX
tctagagtcgaccccgccatgcagcgcgtgaacatgatcatggcagaatcaccaggcctcatcaccatctgccttttaggatatctactcagtgctgaatgtacagtttttcttgatcatgaaaacgccaacaaaattctgaatcggccaaagaggtataattcaggtaaattggaagagtttgttcaagggaaccttgagagagaatgtatggaagaaaagtgtagttttgaagaagcacgagaagtttttgaaaacactgaaagaacaactgaattttggaagcagtatgttgatggagatcagtgtgagtccaatccatgtttaaatggcggcagttgcaaggatgacattaattcctatgaatgttggtgtccctttggatttgaaggaaagaactgtgaattagatgtaacatgtaacattaagaatggcagatgcgagcagttttgtaaaaatagtgctgataacaaggtggtttgctcctgtactgagggatatcgacttgcagaaaaccagaagtcctgtgaaccagcagtgccatttccatgtggaagagtttctgtttcacaaacttctaagctcacccgtgctgaggcagtttttcctgatgtggactatgtaaattctactgaagctgaaaccattttggataacatcactcaaagcacccaatcatttaatgacttcactcgagttgttggtggagaagatgccaaaccaggtcaattcccttggcaggttgttttgaatggtaaagttgatgcattctgtggaggctctatcgttaatgaaaaatggattgtaactgctgcccactgtgttgaaactggtgttaaaattacagttgtcgcaggtgaacataatattgaggagacagaacatacagagcaaaagcgaaatgtgattcgaattattcctcaccacaactacaatgcagctattaataagtacaaccatgacattgcccttctggaactggacgaacccttagtgctaaacagctacgttacacctatttgcattgctgacaaggaatacacgaacatcttcctcaaatttggatctggctatgtaagtggctggggaagagtcttccacaaagggagatcagctttagttcttcagtaccttagagttccacttgttgaccgagccacatgtcttcgatctacaaagttcaccatctataacaacatgttctgtgctggcttccatgaaggaggtagagattcatgtcaaggagatagtgggggaccccatgttactgaagtggaagggaccagtttcttaactggaattattagctggggtgaagagtgtgcaatgaaaggcaaatatggaatatataccaaggtatcccggtatgtcaactggattaaggaaaaaacaaagctcactagctccagcagcaaggcccctcccccgagcctgccctccccaagcaggctgcctgggccctctgacacccctatcctgcctcagtccagctcctctaaggccccaccaccttccctgcctagcccttcaagactgccaggccctagcgatacaccaattctgccccagtcctccagcagcaaggctcccccacctagcctgccttctccatcaaggctgcctggcccatccgataccccaattttgcctcagagcagctctagcaaggcacctccccccagtctgccctctccaagcagactccctggcccttcagacactcccattctgccacagtgatgaggatccgcggccgc

SEQ ID NO: 33 - protein, 583 aa, Artificial Sequence
  CTP-modified Factor IX
SRVDPAMQRVNMIMAESPGLITICLLGYLLSAECTVFLDHENANKILNRPKRYNSGKLEEFVQGNLERECMEEKCSFEEAREVFENTERTTEFWKQYVDGDQCESNPCLNGGSCKDDINSYECWCPFGFEGKNCELDVTCNIKNGRCEQFCKNSADNKVVCSCTEGYRLAENQKSCEPAVPFPCGRVSVSQTSKLTRAEAVFPDVDYVNSTEAETILDNITQSTQSFNDFTRVVGGEDAKPGQFPWQVVLNGKVDAFCGGSIVNEKWIVTAAHCVETGVKITVVAGEHNIEETEHTEQKRNVIRIIPHHNYNAAINKYNHDIALLELDEPLVLNSYVTPICIADKEYTNIFLKFGSGYVSGWGRVFHKGRSALVLQYLRVPLVDRATCLRSTKFTIYNNMFCAGFHEGGRDSCQGDSGGPHVTEVEGTSFLTGIISWGEECAMKGKYGIYTKVSRYVNWIKEKTKLTSSSSKAPPPSLPSPSRLPGPSDTPILPQSSSSKAPPPSLPSPSRLPGPSDTPILPQSSSSKAPPPSLPSPSRLPGPSDTPILPQSSSSKAPPPSLPSPSRLPGPSDTPILPQGSAA

SEQ ID NO: 34 - DNA, 1840 bp, Artificial Sequence
  CTP-modified Factor IX
ctagagtcgaccccgccatgcagcgcgtgaacatgatcatggcagaatcaccaggcctcatcaccatctgccttttaggatatctactcagtgctgaatgtacagtttttcttgatcatgaaaacgccaacaaaattctgaatcggccaaagaggtataattcaggtaaattggaagagtttgttcaagggaaccttgagagagaatgtatggaagaaaagtgtagttttgaagaagcacgagaagtttttgaaaacactgaaagaacaactgaattttggaagcagtatgttgatggagatcagtgtgagtccaatccatgtttaaatggcggcagttgcaaggatgacattaattcctatgaatgttggtgtccctttggatttgaaggaaagaactgtgaattagatgtaacatgtaacattaagaatggcagatgcgagcagttttgtaaaaatagtgctgataacaaggtggtttgctcctgtactgagggatatcgacttgcagaaaaccagaagtcctgtgaaccagcagtgccatttccatgtggaagagtttctgtttcacaaacttctaagctcacccgtgctgaggcagtttttcctgatgtggactatgtaaattctactgaagctgaaaccattttggataacatcactcaaagcacccaatcatttaatgacttcactcgagttgttggtggagaagatgccaaaccaggtcaattcccttggcaggttgttttgaatggtaaagttgatgcattctgtggaggctctatcgttaatgaaaaatggattgtaactgctgcccactgtgttgaaactggtgttaaaattacagttgtcgcaggtgaacataatattgaggagacagaacatacagagcaaaagcgaaatgtgattcgaattattcctcaccacaactacaatgcagctattaataagtacaaccatgacattgcccttctggaactggacgaacccttagtgctaaacagctacgttacacctatttgcattgctgacaaggaatacacgaacatcttcctcaaatttggatctggctatgtaagtggctggggaagagtcttccacaaagggagatcagctttagttcttcagtaccttagagttccacttgttgaccgagccacatgtcttcgatctacaaagttcaccatctataacaacatgttctgtgctggcttccatgaaggaggtagagattcatgtcaaggagatagtgggggaccccatgttactgaagtggaagggaccagtttcttaactggaattattagctggggtgaagagtgtgcaatgaaaggcaaatatggaatatataccaaggtatcccggtatgtcaactggattaaggaaaaaacaaagctcactagctccagcagcaaggcccctcccccgagcctgccctccccaagcaggctgcctgggccctctgacacccctatcctgcctcagtccagctcctctaaggctccaccaccttccctgcctagcccttcaagactgccaggccctagcgatacaccaattctgccccagtcctccagcagcaaggctcccccacctagcctgccttctccatcaaggctgcctggcccatccgataccccaattttgcctcagagcagctctagcaaggcacctccccccagtctgccctctccaagcagactccctggcccttcagacactccaatcctcccacagtcctctagctctaaagctccacctcccagcctgcccagccctagtagactccccggaccttctgatacccccatcttgccccagtgatgaggatccgcggccgc

SEQ ID NO: 35 - protein, 610 aa, Artificial Sequence [sequence omitted]

SEQ ID NO: 36 - DNA, 20 bp, Artificial Sequence
  Primer 101 for FIX-(CTP)2
gtttagtgaaccgtcagaat

SEQ ID NO: 37 - DNA, 20 bp, Artificial Sequence
  Primer 103-R for FIX-(CTP)2
ttgaggaagatgttcgtgta

SEQ ID NO: 38 - DNA, 20 bp, Artificial Sequence
  Primer 98 for FIX-(CTP)2
attacagttgtcgcaggtga

SEQ ID NO: 39 - DNA, 30 bp, Artificial Sequence
  Primer 99-Rfor FIX-(CTP)2
gctggagctagtgagctttgttttttcctt

SEQ ID NO: 40 - DNA, 25 bp, Artificial Sequence
  Primer 100 for FIX-(CTP)2
gctcactagctccagcagcaaggcc

SEQ ID NO: 41 - DNA, 23 bp, Artificial Sequence
  Primer 27-R for FIX-(CTP)2
ttttcactgcattctagttgtgg

SEQ ID NO: 42 - DNA, 20 bp, Artificial Sequence
  Primer 75
ctcccagttcaattacagct

SEQ ID NO: 43 - DNA, 27 bp, Artificial Sequence
  Primer 122r
ggaaaaactgcctcagcacgggtgagc

SEQ ID NO: 44 - DNA, 32 bp, Artificial Sequence
  Primer 123
gtgctgaggcagtttttcctgatgtggactat

SEQ ID NO: 45 - DNA, 18 bp, Artificial Sequence
  Primer 124r
caacacagtgggcagcag